European Patent Specification EP 4 157 311 B1, published June 25, 2025. Title: COMPLEXE IMMUNOMODULATEUR ET SES APPLICATIONS POUR LA THÉRAPIE. Applicant: COMMISSARIAT A L'ENERGIE ATOMIQUE ET AUX ENERGIES ALTERNATIVES. The sequence listing filed with the application follows.

SEQUENCE LISTING (23 sequences)

SEQ ID NO: 1 - protein, 116 aa, artificial sequence
  synthetic polypeptide (BB fragment of Staphylococcus aureus protein A)
ADNKFNKEQQNAFYEILHLPNLNEEQRNGFIQSLKDDPSQSANLLAEAKKLNDAQAPKADNKFNKEQQNAFYEILHLPNLNEEQRNGFIQSLKDDPSQSANLLAEAKKLNDAQAPK

SEQ ID NO: 2 - protein, 116 aa, artificial sequence
  synthetic polypeptide (ZZ derivative of BB fragment of Staphylococcus aureus protein A)
VDNKFNKEQQNAFYEILHLPNLNEEQRNAFIQSLKDDPSQSANLLAEAKKLNDAQAPKVDNKFNKEQQNAFYEILHLPNLNEEQRNAFIQSLKDDPSQSANLLAEAKKLNDAQAPK

SEQ ID NO: 3 - protein, 9 aa, artificial sequence
  synthetic peptide (HIV Tat 49-57)
RKKRRQRRR

SEQ ID NO: 4 - protein, 11 aa, artificial sequence
  synthetic peptide (HIV Tat 28-48)
FTKKGLGISYG

SEQ ID NO: 5 - protein, 154 aa, artificial sequence
  synthetic polypeptide (R domain of Diphteria Toxin)
PGHKTQPFLHDGYAVSWNTVEDSIIRTGFQGESGHDIKITAENTPLPIAGVLLPTIPGKLDVNKSKTHISVNGRKIRMRCRAIDGDVTFCRPKSPVYVGNGVHANLHVAFHRSSSEKIHSNEISSDSIGVLGYQKTVDHTKVNSKLSLFFEIKS

SEQ ID NO: 6 - protein, 16 aa, artificial sequence
  synthetic peptide (penetratin 43-58)
RQIKIWFQNRRMKWKK

SEQ ID NO: 7 - protein, 15 aa, artificial sequence
  synthetic peptide (Diphteria Toxin 453-467)
NGRKIRMRCRAIDGD

SEQ ID NO: 8 - protein, 21 aa, artificial sequence
  synthetic ppetide (HIV Tat 37-57)
CFTKKGLGISYGRKKRRQRRR

SEQ ID NO: 9 - protein, 36 aa, artificial sequence
  synthetic peptide (HIV Tat22-57C (22-37)S)
SNNSYSKKSSFHSQVSFTKKGLGISYGRKKRRQRRR

SEQ ID NO: 10 - protein, 101 aa, artificial sequence
  synthetic polypeptide (HIV Tat consensus sequence)
MEPVDPKLEPWKHPGSQPKTACNNCYCKKCCFHCQVCFTKKGLGISYGRKKRRQRRRAPQDSQTHQVSLSKQPASQPRGDPTGPKESKKKVERETETDPVD

SEQ ID NO: 11 - DNA, 873 bp, artificial sequence
  synthetic polypeptide (ZZ-DTRBDcoli)
atggcgcaacacgatgaagccgtagacaacaaattcaacaaagaacaacaaaacgcgttctatgagatcttacatttacctaacttaaacgaagaacaacgaaacgccttcatccaaagtttaaaagatgacccaagccaaagcgctaaccttttagcagaagctaaaaagctaaatgatgctcaggcgccgaaagtagacaacaaattcaacaaagaacaacaaaacgcgttctatgagatcttacatttacctaacttaaacgaagaacaacgaaacgccttcatccaaagtttaaaagatgacccaagccaaagcgctaaccttttagcagaagctaaaaagctaaatgatgctcaggcgccgaaagtagacgcgaattcgagctcggtaccgtcgacgccgggtcataaaacccagccgtttctgcatgatggctatgcggtgagctggaacaccgtggaagatagcattattcgtaccggctttcagggcgaaagcggccatgatattaaaattaccgcggaaaacaccccgctgccgattgcgggtgttctgctgccgaccattccgggcaaactggatgtgaacaaaagcaaaacccatattagcgtgaacggccgtaaaattcgtatgcgttgccgtgcgattgatggtgatgtgaccttttgccgtccgaaaagcccggtgtatgtgggcaacggcgtgcatgcgaacctgcatgtggcgtttcatcgtagcagcagcgaaaaaatccatagcaacgaaattagcagcgatagcattggcgtgctgggctatcagaaaaccgtggatcataccaaagtgaactctaaactgagcctgttcttcgaaatcaaaagcggaagctta

SEQ ID NO: 12 - protein, 291 aa, artificial sequence
  synthetic polypeptide (ZZ-DTRBDcoli)
MAQHDEAVDNKFNKEQQNAFYEILHLPNLNEEQRNAFIQSLKDDPSQSANLLAEAKKLNDAQAPKVDNKFNKEQQNAFYEILHLPNLNEEQRNAFIQSLKDDPSQSANLLAEAKKLNDAQAPKVDANSSSVPSTPGHKTQPFLHDGYAVSWNTVEDSIIRTGFQGESGHDIKITAENTPLPIAGVLLPTIPGKLDVNKSKTHISVNGRKIRMRCRAIDGDVTFCRPKSPVYVGNGVHANLHVAFHRSSSEKIHSNEISSDSIGVLGYQKTVDHTKVNSKLSLFFEIKSGSL

SEQ ID NO: 13 - DNA, 930 bp, artificial sequence
  synthetic polynucleotide (ZZ-DTRBDHEK )
atgggctggtcctgcatcatcctgtttctggtggccacagccaccggtgttcactctgcccagcatgatgaggccgtggacaacaagttcaacaaagagcagcagaacgccttctacgagatcctgcatctgcccaacctgaacgaggaacagagaaacgccttcatccagagcctgaaggacgaccctagccagagcgctaatctgctggccgaggccaagaagctgaacgacgctcaggcccctaaagtcgataacaagtttaacaaagaacaacaaaatgccttttatgagatcctccaccttccgaatctcaatgaggaacagcggaatgcctttattcagtccctgaaggatgatccctctcagtccgccaacctgctggctgaagctaaaaaactgaatgatgcccaggctcctaaggtggacgcgaatgctagcagcggggtaccctcaacaccagggcacaagactcagcccttcctgcacgatggctatgctgtgagctggaatacagtggaagattccatcattaggacaggctttcaaggcgaaagtggccatgacatcaagattactgccgaaaacaccccattgccgatagctggtgttctccttcccacgattcctgggaaactggacgtcaacaagtccaagactcacatctccgtgaatggacgcaaaatacggatgcgatgtagagccattgatggcgatgtgaccttttgcagacccaaatctcctgtgtacgttgggaatgtaggtcatgcgaatctccatgtcgcatttcaccgttcatcctctgagaagatccacagcaacgagatcagctctgactcaattggagtgctgggataccagaaaaccgtagaccataccaaggtcaacagcaagctgagtctgttcttcgagatcaaaagcggaagctta

SEQ ID NO: 14 - protein, 291 aa, artificial sequence
  synthetic polypeptide (ZZ-DTRBDHEK)
AQHDEAVDNKFNKEQQNAFYEILHLPNLNEEQRNAFIQSLKDDPSQSANLLAEAKKLNDAQAPKVDNKFNKEQQNAFYEILHLPNLNEEQRNAFIQSLKDDPSQSANLLAEAKKLNDAQAPKVDANASSGVPSTPGHKTQPFLHDGYAVSWNTVEDSIIRTGFQGESGHDIKITAENTPLPIAGVLLPTIPGKLDVNKSKTHISVNGRKIRMRCRAIDGDVTFCRPKSPVYVGNVGHANLHVAFHRSSSEKIHSNEISSDSIGVLGYQKTVDHTKVNSKLSLFFEIKSGSL

SEQ ID NO: 15 - DNA, 873 bp, artificial sequence
  synthetic polynucleotide (BB-DTRBDcoli)
atggcgcaacacgatgaagccgcagacaacaaattcaacaaagaacaacaaaacgcgttctatgagatcttacatttacctaacttaaacgaagaacaacgaaacggtttcatccaaagtttaaaagatgacccaagccaaagcgctaaccttttagcagaagctaaaaagctaaatgatgctcaggcgccgaaagcagacaacaaattcaacaaagaacaacaaaacgcgttctatgagatcttacatttacctaacttaaacgaagaacaacgaaacggtttcatccaaagtttaaaagatgacccaagccaaagcgctaaccttttagcagaagctaaaaagctaaatgatgctcaggcgccgaaagtagacgcgaattcgagctcggtaccgtcgacgccgggtcataaaacccagccgtttctgcatgatggctatgcggtgagctggaacaccgtggaagatagcattattcgtaccggctttcagggcgaaagcggccatgatattaaaattaccgcggaaaacaccccgctgccgattgcgggtgttctgctgccgaccattccgggcaaactggatgtgaacaaaagcaaaacccatattagcgtgaacggccgtaaaattcgtatgcgttgccgtgcgattgatggtgatgtgaccttttgccgtccgaaaagcccggtgtatgtgggcaacggcgtgcatgcgaacctgcatgtggcgtttcatcgtagcagcagcgaaaaaatccatagcaacgaaattagcagcgatagcattggcgtgctgggctatcagaaaaccgtggatcataccaaagtgaactctaaactgagcctgttcttcgaaatcaaaagcggaagctta

SEQ ID NO: 16 - protein, 291 aa, artificial sequence
  synthetic polypeptide (BB-DTRBDcoli)
MAQHDEAADNKFNKEQQNAFYEILHLPNLNEEQRNGFIQSLKDDPSQSANLLAEAKKLNDAQAPKADNKFNKEQQNAFYEILHLPNLNEEQRNGFIQSLKDDPSQSANLLAEAKKLNDAQAPKVDANSSSVPSTPGHKTQPFLHDGYAVSWNTVEDSIIRTGFQGESGHDIKITAENTPLPIAGVLLPTIPGKLDVNKSKTHISVNGRKIRMRCRAIDGDVTFCRPKSPVYVGNGVHANLHVAFHRSSSEKIHSNEISSDSIGVLGYQKTVDHTKVNSKLSLFFEIKSGSL

SEQ ID NO: 17 - DNA, 930 bp, artificial sequence
  synthetic polynucleotide (BB-DTRBDHEK)
atgggctggtcctgcatcatcctgtttctggtggccacagccaccggtgttcactctgcccagcatgatgaggccgccgacaacaagttcaacaaagagcagcagaacgccttctacgagatcctgcatctgcccaacctgaacgaggaacagagaaacggcttcatccagagcctgaaggacgaccctagccagagcgctaatctgctggccgaggccaagaagctgaacgacgctcaggcccctaaagccgataacaagtttaacaaagaacaacaaaatgccttttatgagatcctccaccttccgaatctcaatgaggaacagcggaatggctttattcagtccctgaaggatgatccctctcagtccgccaacctgctggctgaagctaaaaaactgaatgatgcccaggctcctaaggtggacgcgaatgctagcagcggggtaccctcaacaccagggcacaagactcagcccttcctgcacgatggctatgctgtgagctggaatacagtggaagattccatcattaggacaggctttcaaggcgaaagtggccatgacatcaagattactgccgaaaacaccccattgccgatagctggtgttctccttcccacgattcctgggaaactggacgtcaacaagtccaagactcacatctccgtgaatggacgcaaaatacggatgcgatgtagagccattgatggcgatgtgaccttttgcagacccaaatctcctgtgtacgttgggaatgtaggtcatgcgaatctccatgtcgcatttcaccgttcatcctctgagaagatccacagcaacgagatcagctctgactcaattggagtgctgggataccagaaaaccgtagaccataccaaggtcaacagcaagctgagtctgttcttcgagatcaaaagcggaagctta

SEQ ID NO: 18 - protein, 291 aa, artificial sequence
  synthetic polypeptide (BB-DTRBDHEK)
AQHDEAADNKFNKEQQNAFYEILHLPNLNEEQRNGFIQSLKDDPSQSANLLAEAKKLNDAQAPKADNKFNKEQQNAFYEILHLPNLNEEQRNGFIQSLKDDPSQSANLLAEAKKLNDAQAPKVDANASSGVPSTPGHKTQPFLHDGYAVSWNTVEDSIIRTGFQGESGHDIKITAENTPLPIAGVLLPTIPGKLDVNKSKTHISVNGRKIRMRCRAIDGDVTFCRPKSPVYVGNVGHANLHVAFHRSSSEKIHSNEISSDSIGVLGYQKTVDHTKVNSKLSLFFEIKSGSL

SEQ ID NO: 19 - DNA, 504 bp, artificial sequence
  synthetic polynucleotide (ZZ-Tat22-57C(22-37)Scoli )
atggcgcaacacgatgaagccgtagacaacaaattcaacaaagaacaacaaaacgcgttctatgagatcttacatttacctaacttaaacgaagaacaacgaaacgccttcatccaaagtttaaaagatgacccaagccaaagcgctaaccttttagcagaagctaaaaagctaaatgatgctcaggcgccgaaagtagacaacaaattcaacaaagaacaacaaaacgcgttctatgagatcttacatttacctaacttaaacgaagaacaacgaaacgccttcatccaaagtttaaaagatgacccaagccaaagcgctaaccttttagcagaagctaaaaagctaaatgatgctcaggcgccgaaagtagacgcgaattcgagctcggtacccagcaataattcctatagcaaaaaaagcagctttcatagccaggtgagctttaccaaaaaaggcctgggcattagctatggccgtaaaaaacgtcgtcagcgtcgtcgt

SEQ ID NO: 20 - protein, 168 aa, artificial sequence
  synthetic polypeptide (ZZ-Tat22-57C(22-37)Scoli )
MAQHDEAVDNKFNKEQQNAFYEILHLPNLNEEQRNAFIQSLKDDPSQSANLLAEAKKLNDAQAPKVDNKFNKEQQNAFYEILHLPNLNEEQRNAFIQSLKDDPSQSANLLAEAKKLNDAQAPKVDANSSSVPSNNSYSKKSSFHSQVSFTKKGLGISYGRKKRRQRRR

SEQ ID NO: 21 - protein, 11 aa, artificial sequence
  synthetic peptide (linker)
VDANSSSVPST

SEQ ID NO: 22 - protein, 12 aa, artificial sequence
  synthetic peptide (linker)
VDANASSGVPST

SEQ ID NO: 23 - protein, 9 aa, artificial sequence
  synthetic peptide (linker)
VDANSSSVP